European Patent Application EP 4 667 480 A1, published December 24, 2025. Title: Translation initiation with exotic amino acids using EF-P-responsive artificial initiator tRNA. Applicant: The University of Tokyo. The sequence listing filed with the application follows.

SEQUENCE LISTING (248 sequences)

SEQ ID NO: 1-8 - skipped (8 entries)

SEQ ID NO: 9 - RNA, 17 nt, synthetic construct
  misc_feature 1..17: note = D-arm of initiator tRNA
  source 1..17: mol_type = other RNA
gcgcagcctggtagcgc

SEQ ID NO: 10-11 - skipped (2 entries)

SEQ ID NO: 12 - RNA, 18 nt, synthetic construct
  misc_feature 1..18: note = anticodon stem and anticodon loop of initiator tRNA
  misc_feature 7..13: note = n is a, c, g, or u
  source 1..18: mol_type = other RNA
gtcgggnnnnnnncccga

SEQ ID NO: 13 - RNA, 18 nt, synthetic construct
  misc_feature 1..18: note = anticodon stem and anticodon loop of initiator tRNA
  misc_feature 7..13: note = n is a, c, g, or u
  source 1..18: mol_type = other RNA
atcgggnnnnnnncccga

SEQ ID NO: 14 - RNA, 18 nt, synthetic construct
  misc_feature 1..18: note = anticodon stem and anticodon loop of initiator tRNA
  misc_feature 7..13: note = n is a, c, g, or u
  source 1..18: mol_type = other RNA
accgggnnnnnnncccgg

SEQ ID NO: 15 - RNA, 18 nt, synthetic construct
  misc_feature 1..18: note = anticodon stem and anticodon loop of initiator tRNA
  misc_feature 7..13: note = n is a, c, g, or u
  source 1..18: mol_type = other RNA
actgggnnnnnnncccag

SEQ ID NO: 16 - RNA, 18 nt, synthetic construct
  misc_feature 1..18: note = anticodon stem and anticodon loop of initiator tRNA
  misc_feature 7..13: note = n is a, c, g, or u
  source 1..18: mol_type = other RNA
acttggnnnnnnnccaag

SEQ ID NO: 17 - skipped

SEQ ID NO: 18 - RNA, 18 nt, synthetic construct
  misc_feature 1..18: note = anticodon stem and anticodon loop of initiator tRNA
  misc_feature 9..11: note = n is a, c, g, or u
  source 1..18: mol_type = other RNA
gtcgggctnnnaacccga

SEQ ID NO: 19 - RNA, 18 nt, synthetic construct
  misc_feature 1..18: note = anticodon stem and anticodon loop of initiator tRNA
  misc_feature 9..11: note = n is a, c, g, or u
  source 1..18: mol_type = other RNA
atcgggctnnnaacccga

SEQ ID NO: 20 - RNA, 18 nt, synthetic construct
  misc_feature 1..18: note = anticodon stem and anticodon loop of initiator tRNA
  misc_feature 9..11: note = n is a, c, g, or u
  source 1..18: mol_type = other RNA
accgggctnnnaacccgg

SEQ ID NO: 21 - RNA, 18 nt, synthetic construct
  misc_feature 1..18: note = anticodon stem and anticodon loop of initiator tRNA
  misc_feature 9..11: note = n is a, c, g, or u
  source 1..18: mol_type = other RNA
actgggctnnnaacccag

SEQ ID NO: 22 - RNA, 18 nt, synthetic construct
  misc_feature 1..18: note = anticodon stem and anticodon loop of initiator tRNA
  misc_feature 9..11: note = n is a, c, g, or u
  source 1..18: mol_type = other RNA
acttggctnnnaaccaag

SEQ ID NO: 23 - skipped

SEQ ID NO: 24 - RNA, 17 nt, synthetic construct
  misc_feature 1..17: note = T-arm of initiator tRNA
  source 1..17: mol_type = other RNA
gtcggttcaaatccggc

SEQ ID NO: 25 - RNA, 17 nt, synthetic construct
  misc_feature 1..17: note = T-arm of initiator tRNA
  source 1..17: mol_type = other RNA
gtcggttcaaatccggt

SEQ ID NO: 26 - RNA, 17 nt, synthetic construct
  misc_feature 1..17: note = T-arm of initiator tRNA
  source 1..17: mol_type = other RNA
ggcggttcaaatccgct

SEQ ID NO: 27 - RNA, 17 nt, synthetic construct
  misc_feature 1..17: note = T-arm of initiator tRNA
  source 1..17: mol_type = other RNA
ggaggttcaaatcctct

SEQ ID NO: 28-31 - skipped (4 entries)

SEQ ID NO: 32 - RNA, 46 nt, synthetic construct
  misc_feature 1..46: note = RNA sequence of dFx
  source 1..46: mol_type = other RNA
ggatcgaaagatttccgcatccccgaaagggtacatggcgttaggt

SEQ ID NO: 33 - RNA, 45 nt, synthetic construct
  misc_feature 1..45: note = RNA sequence of eFx
  source 1..45: mol_type = other RNA
ggatcgaaagatttccgcggccccgaaaggggattagcgttaggt

SEQ ID NO: 34 - DNA, 36 bp, synthetic construct
  misc_feature 1..36: note = Extension primer (forward) of dFx
  source 1..36: mol_type = other DNA
gtaatacgactcactataggatcgaaagatttccgc

SEQ ID NO: 35 - DNA, 36 bp, synthetic construct; identical to SEQ ID NO: 34
  misc_feature 1..36: note = Extension primer (forward) of eFx
  source 1..36: mol_type = other DNA

SEQ ID NO: 36 - DNA, 46 bp, synthetic construct
  misc_feature 1..46: note = Extension primer (reverse) of dFx
  source 1..46: mol_type = other DNA
acctaacgccatgtaccctttcggggatgcggaaatctttcgatcc

SEQ ID NO: 37 - DNA, 45 bp, synthetic construct
  misc_feature 1..45: note = Extension primer (reverse) of eFx
  source 1..45: mol_type = other DNA
acctaacgctaatcccctttcggggccgcggaaatctttcgatcc

SEQ ID NO: 38 - DNA, 22 bp, synthetic construct
  misc_feature 1..22: note = PCR primer (forward) of dFx
  source 1..22: mol_type = other DNA
ggcgtaatacgactcactatag

SEQ ID NO: 39 - DNA, 22 bp, synthetic construct
  misc_feature 1..22: note = PCR primer (forward) of eFx
  source 1..22: mol_type = other DNA
ggcgtaatacgactcactatag

SEQ ID NO: 40 - DNA, 19 bp, synthetic construct
  misc_feature 1..19: note = PCR primer (reverse) of dFx
  source 1..19: mol_type = other DNA
acctaacgccatgtaccct

SEQ ID NO: 41 - DNA, 18 bp, synthetic construct
  misc_feature 1..18: note = PCR primer (reverse) of eFx
  source 1..18: mol_type = other DNA
acctaacgctaatcccct

SEQ ID NO: 42 - RNA, 77 nt, synthetic construct
  misc_feature 1..77: note = RNA sequence of tRNA, iniWT
  source 1..77: mol_type = other RNA
cgcggggtggagcagcctggtagctcgtcgggctcataacccgaagatcgtcggttcaaatccggcccccgcaacca

SEQ ID NO: 43 - RNA, 77 nt, synthetic construct
  misc_feature 1..77: note = RNA sequence of tRNA, iniC1G
  source 1..77: mol_type = other RNA
ggcggggtggagcagcctggtagctcgtcgggctcataacccgaagatcgtcggttcaaatccggcccccgcaacca

SEQ ID NO: 44 - RNA, 77 nt, synthetic construct
  misc_feature 1..77: note = RNA sequence of tRNA, An1Ac1T1V1 (=iniC1G/A11C/U24G)
  source 1..77: mol_type = other RNA
ggcggggtggcgcagcctggtagcgcgtcgggctcataacccgaagatcgtcggttcaaatccggcccccgcaacca

SEQ ID NO: 45 - RNA, 77 nt, synthetic construct
  misc_feature 1..77: note = RNA sequence of tRNA, An2Ac1T1V1
  source 1..77: mol_type = other RNA
ggcggggtggcgcagcctggtagcgcatcgggctcataacccgaagatcgtcggttcaaatccggcccccgcaacca

SEQ ID NO: 46 - RNA, 77 nt, synthetic construct
  misc_feature 1..77: note = RNA sequence of tRNA, An3Ac1T1V1
  source 1..77: mol_type = other RNA
ggcggggtggcgcagcctggtagcgcaccgggctcataacccggagatcgtcggttcaaatccggcccccgcaacca

SEQ ID NO: 47 - RNA, 77 nt, synthetic construct
  misc_feature 1..77: note = RNA sequence of tRNA, An4Ac1T1V1
  source 1..77: mol_type = other RNA
ggcggggtggcgcagcctggtagcgcactgggctcataacccagagatcgtcggttcaaatccggcccccgcaacca

SEQ ID NO: 48 - RNA, 77 nt, synthetic construct
  misc_feature 1..77: note = RNA sequence of tRNA, An5Ac1T1V1
  source 1..77: mol_type = other RNA
ggcggggtggcgcagcctggtagcgcacttggctcataaccaagagatcgtcggttcaaatccggcccccgcaacca

SEQ ID NO: 49 - RNA, 77 nt, synthetic construct
  misc_feature 1..77: note = RNA sequence of tRNA, An4Ac2T1V1
  source 1..77: mol_type = other RNA
ggcgggttggcgcagcctggtagcgcactgggctcataacccagagatcgtcggttcaaatccggcacccgcaacca

SEQ ID NO: 50 - RNA, 77 nt, synthetic construct
  misc_feature 1..77: note = RNA sequence of tRNA, An4Ac3T1V1
  source 1..77: mol_type = other RNA
ggcggattggcgcagcctggtagcgcactgggctcataacccagagatcgtcggttcaaatccggcatccgcaacca

SEQ ID NO: 51 - RNA, 77 nt, synthetic construct
  misc_feature 1..77: note = RNA sequence of tRNA, An4Ac4T1V1
  source 1..77: mol_type = other RNA
ggctgattggcgcagcctggtagcgcactgggctcataacccagagatcgtcggttcaaatccggcatcagcaacca

SEQ ID NO: 52 - RNA, 77 nt, synthetic construct
  misc_feature 1..77: note = RNA sequence of tRNA, An4Ac5T1V1
  source 1..77: mol_type = other RNA
gggtgattggcgcagcctggtagcgcactgggctcataacccagagatcgtcggttcaaatccggcatcaccaacca

SEQ ID NO: 53 - RNA, 77 nt, synthetic construct
  misc_feature 1..77: note = RNA sequence of tRNA, An4Ac1T1V2
  source 1..77: mol_type = other RNA
ggcggggtggcgcagcctggtagcgcactgggctcataacccagggatcgtcggttcaaatccggcccccgcaacca

SEQ ID NO: 54 - RNA, 77 nt, synthetic construct
  misc_feature 1..77: note = RNA sequence of tRNA, An4Ac1T1V3
  source 1..77: mol_type = other RNA
ggcggggtggcgcagcctggtagcgcactgggctcataacccagaggtcgtcggttcaaatccggcccccgcaacca

SEQ ID NO: 55 - RNA, 77 nt, synthetic construct
  misc_feature 1..77: note = RNA sequence of tRNA, An4Ac1T1V4
  source 1..77: mol_type = other RNA
ggcggggtggcgcagcctggtagcgcactgggctcataacccaggggtcgtcggttcaaatccggcccccgcaacca

SEQ ID NO: 56 - RNA, 77 nt, synthetic construct
  misc_feature 1..77: note = RNA sequence of tRNA, An4Ac1T2V1
  source 1..77: mol_type = other RNA
ggcggggtggcgcagcctggtagcgcactgggctcataacccagagatcgtcggttcaaatccggtccccgcaacca

SEQ ID NO: 57 - RNA, 77 nt, synthetic construct
  misc_feature 1..77: note = RNA sequence of tRNA, An4Ac1T2V2
  source 1..77: mol_type = other RNA
ggcggggtggcgcagcctggtagcgcactgggctcataacccagggatcgtcggttcaaatccggtccccgcaacca

SEQ ID NO: 58 - RNA, 77 nt, synthetic construct
  misc_feature 1..77: note = RNA sequence of tRNA, An4Ac1T2V3
  source 1..77: mol_type = other RNA
ggcggggtggcgcagcctggtagcgcactgggctcataacccagaggtcgtcggttcaaatccggtccccgcaacca

SEQ ID NO: 59 - RNA, 77 nt, synthetic construct
  misc_feature 1..77: note = RNA sequence of tRNA, An4Ac1T2V4
  source 1..77: mol_type = other RNA
ggcggggtggcgcagcctggtagcgcactgggctcataacccaggggtcgtcggttcaaatccggtccccgcaacca

SEQ ID NO: 60 - RNA, 77 nt, synthetic construct
  misc_feature 1..77: note = RNA sequence of tRNA, An4Ac1T3V1
  source 1..77: mol_type = other RNA
ggcggggtggcgcagcctggtagcgcactgggctcataacccagagatcggcggttcaaatccgctccccgcaacca

SEQ ID NO: 61 - RNA, 77 nt, synthetic construct
  misc_feature 1..77: note = RNA sequence of tRNA, An4Ac1T3V2
  source 1..77: mol_type = other RNA
ggcggggtggcgcagcctggtagcgcactgggctcataacccagggatcggcggttcaaatccgctccccgcaacca

SEQ ID NO: 62 - RNA, 77 nt, synthetic construct
  misc_feature 1..77: note = RNA sequence of tRNA, An4Ac1T3V3 (=iniP)
  source 1..77: mol_type = other RNA
ggcggggtggcgcagcctggtagcgcactgggctcataacccagaggtcggcggttcaaatccgctccccgcaacca

SEQ ID NO: 63 - RNA, 77 nt, synthetic construct
  misc_feature 1..77: note = RNA sequence of tRNA, An4Ac1T3V4
  source 1..77: mol_type = other RNA
ggcggggtggcgcagcctggtagcgcactgggctcataacccaggggtcggcggttcaaatccgctccccgcaacca

SEQ ID NO: 64 - RNA, 77 nt, synthetic construct
  misc_feature 1..77: note = RNA sequence of tRNA, An4Ac1T4V1
  source 1..77: mol_type = other RNA
ggcggggtggcgcagcctggtagcgcactgggctcataacccagagatcggaggttcaaatcctctccccgcaacca

SEQ ID NO: 65 - RNA, 77 nt, synthetic construct
  misc_feature 1..77: note = RNA sequence of tRNA, An4Ac1T4V2
  source 1..77: mol_type = other RNA
ggcggggtggcgcagcctggtagcgcactgggctcataacccagggatcggaggttcaaatcctctccccgcaacca

SEQ ID NO: 66 - RNA, 77 nt, synthetic construct
  misc_feature 1..77: note = RNA sequence of tRNA, An4Ac1T4V3
  source 1..77: mol_type = other RNA
ggcggggtggcgcagcctggtagcgcactgggctcataacccagaggtcggaggttcaaatcctctccccgcaacca

SEQ ID NO: 67 - RNA, 77 nt, synthetic construct
  misc_feature 1..77: note = RNA sequence of tRNA, An4Ac1T4V4
  source 1..77: mol_type = other RNA
ggcggggtggcgcagcctggtagcgcactgggctcataacccaggggtcggaggttcaaatcctctccccgcaacca

SEQ ID NO: 68 - RNA, 77 nt, synthetic construct
  misc_feature 1..77: note = RNA sequence of tRNA, An4Ac1T3V3, anticodon=CUU
  source 1..77: mol_type = other RNA
ggcggggtggcgcagcctggtagcgcactgggctcttaacccagaggtcggcggttcaaatccgctccccgcaacca

SEQ ID NO: 69 - DNA, 50 bp, synthetic construct
  misc_feature 1..50: note = Extension primer (forward) of tRNA, iniWT
  source 1..50: mol_type = other DNA
gtaatacgactcactatacgcggggtggagcagcctggtagctcgtcggg

SEQ ID NO: 70 - DNA, 50 bp, synthetic construct
  misc_feature 1..50: note = Extension primer (forward) of tRNA, iniC1G
  source 1..50: mol_type = other DNA
gtaatacgactcactataggcggggtggagcagcctggtagctcgtcggg

SEQ ID NO: 71 - DNA, 45 bp, synthetic construct
  misc_feature 1..45: note = Extension primer (forward) of tRNA, An1Ac1T1V1(=iniC1G/A11C/U24G)
  source 1..45: mol_type = other DNA
gtaatacgactcactataggcggggtggcgcagcctggtagcgcg

SEQ ID NO: 72 - DNA, 45 bp, synthetic construct
  misc_feature 1..45: note = Extension primer (forward) of tRNA, An2Ac1T1V1
  source 1..45: mol_type = other DNA
gtaatacgactcactataggcggggtggcgcagcctggtagcgca

SEQ ID NO: 73 - DNA, 45 bp, synthetic construct; identical to SEQ ID NO: 72
  misc_feature 1..45: note = Extension primer (forward) of tRNA, An3Ac1T1V1
  source 1..45: mol_type = other DNA

SEQ ID NO: 74 - DNA, 45 bp, synthetic construct; identical to SEQ ID NO: 72
  misc_feature 1..45: note = Extension primer (forward) of tRNA, An4Ac1T1V1
  source 1..45: mol_type = other DNA

SEQ ID NO: 75 - DNA, 45 bp, synthetic construct; identical to SEQ ID NO: 72
  misc_feature 1..45: note = Extension primer (forward) of tRNA, An5Ac1T1V1
  source 1..45: mol_type = other DNA

SEQ ID NO: 76 - DNA, 45 bp, synthetic construct
  misc_feature 1..45: note = Extension primer (forward) of tRNA, An4Ac2T1V1
  source 1..45: mol_type = other DNA
gtaatacgactcactataggcgggttggcgcagcctggtagcgca

SEQ ID NO: 77 - DNA, 45 bp, synthetic construct
  misc_feature 1..45: note = Extension primer (forward) of tRNA, An4Ac3T1V1
  source 1..45: mol_type = other DNA
gtaatacgactcactataggcggattggcgcagcctggtagcgca

SEQ ID NO: 78 - DNA, 45 bp, synthetic construct
  misc_feature 1..45: note = Extension primer (forward) of tRNA, An4Ac4T1V1
  source 1..45: mol_type = other DNA
gtaatacgactcactataggctgattggcgcagcctggtagcgca

SEQ ID NO: 79 - DNA, 45 bp, synthetic construct
  misc_feature 1..45: note = Extension primer (forward) of tRNA, An4Ac5T1V1
  source 1..45: mol_type = other DNA
gtaatacgactcactatagggtgattggcgcagcctggtagcgca

SEQ ID NO: 80 - DNA, 45 bp, synthetic construct; identical to SEQ ID NO: 72
  misc_feature 1..45: note = Extension primer (forward) of tRNA, An4Ac1T1V2
  source 1..45: mol_type = other DNA

SEQ ID NO: 81 - DNA, 45 bp, synthetic construct; identical to SEQ ID NO: 72
  misc_feature 1..45: note = Extension primer (forward) of tRNA, An4Ac1T1V3
  source 1..45: mol_type = other DNA

SEQ ID NO: 82 - DNA, 45 bp, synthetic construct; identical to SEQ ID NO: 72
  misc_feature 1..45: note = Extension primer (forward) of tRNA, An4Ac1T1V4
  source 1..45: mol_type = other DNA

SEQ ID NO: 83 - DNA, 45 bp, synthetic construct; identical to SEQ ID NO: 72
  misc_feature 1..45: note = Extension primer (forward) of tRNA, An4Ac1T2V1
  source 1..45: mol_type = other DNA

SEQ ID NO: 84 - DNA, 45 bp, synthetic construct; identical to SEQ ID NO: 72
  misc_feature 1..45: note = Extension primer (forward) of tRNA, An4Ac1T2V2
  source 1..45: mol_type = other DNA

SEQ ID NO: 85 - DNA, 45 bp, synthetic construct; identical to SEQ ID NO: 72
  misc_feature 1..45: note = Extension primer (forward) of tRNA, An4Ac1T2V3
  source 1..45: mol_type = other DNA

SEQ ID NO: 86 - DNA, 45 bp, synthetic construct; identical to SEQ ID NO: 72
  misc_feature 1..45: note = Extension primer (forward) of tRNA, An4Ac1T2V4
  source 1..45: mol_type = other DNA

SEQ ID NO: 87 - DNA, 45 bp, synthetic construct; identical to SEQ ID NO: 72
  misc_feature 1..45: note = Extension primer (forward) of tRNA, An4Ac1T3V1
  source 1..45: mol_type = other DNA

SEQ ID NO: 88 - DNA, 45 bp, synthetic construct; identical to SEQ ID NO: 72
  misc_feature 1..45: note = Extension primer (forward) of tRNA, An4Ac1T3V2
  source 1..45: mol_type = other DNA

SEQ ID NO: 89 - DNA, 45 bp, synthetic construct; identical to SEQ ID NO: 72
  misc_feature 1..45: note = Extension primer (forward) of tRNA, An4Ac1T3V3 (=iniP)
  source 1..45: mol_type = other DNA

SEQ ID NO: 90 - DNA, 45 bp, synthetic construct; identical to SEQ ID NO: 72
  misc_feature 1..45: note = Extension primer (forward) of tRNA, An4Ac1T3V4
  source 1..45: mol_type = other DNA

SEQ ID NO: 91 - DNA, 45 bp, synthetic construct; identical to SEQ ID NO: 72
  misc_feature 1..45: note = Extension primer (forward) of tRNA, An4Ac1T4V1
  source 1..45: mol_type = other DNA

SEQ ID NO: 92 - DNA, 45 bp, synthetic construct; identical to SEQ ID NO: 72
  misc_feature 1..45: note = Extension primer (forward) of tRNA, An4Ac1T4V2
  source 1..45: mol_type = other DNA

SEQ ID NO: 93 - DNA, 45 bp, synthetic construct; identical to SEQ ID NO: 72
  misc_feature 1..45: note = Extension primer (forward) of tRNA, An4Ac1T4V3
  source 1..45: mol_type = other DNA

SEQ ID NO: 94 - DNA, 45 bp, synthetic construct; identical to SEQ ID NO: 72
  misc_feature 1..45: note = Extension primer (forward) of tRNA, An4Ac1T4V4
  source 1..45: mol_type = other DNA

SEQ ID NO: 95 - DNA, 45 bp, synthetic construct; identical to SEQ ID NO: 72
  misc_feature 1..45: note = Extension primer (forward) of tRNA, An4Ac1T3V3, anticodon=CUU
  source 1..45: mol_type = other DNA

SEQ ID NO: 96 - DNA, 62 bp, synthetic construct
  misc_feature 1..62: note = Extension primer (reverse) of tRNA, iniWT
  source 1..62: mol_type = other DNA
tggttgcgggggccggatttgaaccgacgatcttcgggttatgagcccgacgagctaccagg

SEQ ID NO: 97 - DNA, 62 bp, synthetic construct; identical to SEQ ID NO: 96
  misc_feature 1..62: note = Extension primer (reverse) of tRNA, iniC1G
  source 1..62: mol_type = other DNA

SEQ ID NO: 98 - DNA, 68 bp, synthetic construct
  misc_feature 1..68: note = Extension primer (reverse) of tRNA, An1Ac1T1V1(=iniC1G/A11C/U24G)
  source 1..68: mol_type = other DNA
tggttgcgggggccggatttgaaccgacgatcttcgggttatgagcccgacgcgctaccaggctgcgc

SEQ ID NO: 99 - DNA, 68 bp, synthetic construct
  misc_feature 1..68: note = Extension primer (reverse) of tRNA, An2Ac1T1V1
  source 1..68: mol_type = other DNA
tggttgcgggggccggatttgaaccgacgatcttcgggttatgagcccgatgcgctaccaggctgcgc

SEQ ID NO: 100 - DNA, 68 bp, synthetic construct
  misc_feature 1..68: note = Extension primer (reverse) of tRNA, An3Ac1T1V1
  source 1..68: mol_type = other DNA
tggttgcgggggccggatttgaaccgacgatctccgggttatgagcccggtgcgctaccaggctgcgc

SEQ ID NO: 101 - DNA, 68 bp, synthetic construct
  misc_feature 1..68: note = Extension primer (reverse) of tRNA, An4Ac1T1V1
  source 1..68: mol_type = other DNA
tggttgcgggggccggatttgaaccgacgatctctgggttatgagcccagtgcgctaccaggctgcgc

SEQ ID NO: 102 - DNA, 68 bp, synthetic construct
  misc_feature 1..68: note = Extension primer (reverse) of tRNA, An5Ac1T1V1
  source 1..68: mol_type = other DNA
tggttgcgggggccggatttgaaccgacgatctcttggttatgagccaagtgcgctaccaggctgcgc

SEQ ID NO: 103 - DNA, 68 bp, synthetic construct
  misc_feature 1..68: note = Extension primer (reverse) of tRNA, An4Ac2T1V1
  source 1..68: mol_type = other DNA
tggttgcgggtgccggatttgaaccgacgatctctgggttatgagcccagtgcgctaccaggctgcgc

SEQ ID NO: 104 - DNA, 68 bp, synthetic construct
  misc_feature 1..68: note = Extension primer (reverse) of tRNA, An4Ac3T1V1
  source 1..68: mol_type = other DNA
tggttgcggatgccggatttgaaccgacgatctctgggttatgagcccagtgcgctaccaggctgcgc

SEQ ID NO: 105 - DNA, 68 bp, synthetic construct
  misc_feature 1..68: note = Extension primer (reverse) of tRNA, An4Ac4T1V1
  source 1..68: mol_type = other DNA
tggttgctgatgccggatttgaaccgacgatctctgggttatgagcccagtgcgctaccaggctgcgc

SEQ ID NO: 106 - DNA, 68 bp, synthetic construct
  misc_feature 1..68: note = Extension primer (reverse) of tRNA, An4Ac5T1V1
  source 1..68: mol_type = other DNA
tggttggtgatgccggatttgaaccgacgatctctgggttatgagcccagtgcgctaccaggctgcgc

SEQ ID NO: 107 - DNA, 68 bp, synthetic construct
  misc_feature 1..68: note = Extension primer (reverse) of tRNA, An4Ac1T1V2
  source 1..68: mol_type = other DNA
tggttgcgggggccggatttgaaccgacgatccctgggttatgagcccagtgcgctaccaggctgcgc

SEQ ID NO: 108 - DNA, 68 bp, synthetic construct
  misc_feature 1..68: note = Extension primer (reverse) of tRNA, An4Ac1T1V3
  source 1..68: mol_type = other DNA
tggttgcgggggccggatttgaaccgacgacctctgggttatgagcccagtgcgctaccaggctgcgc

SEQ ID NO: 109 - DNA, 68 bp, synthetic construct
  misc_feature 1..68: note = Extension primer (reverse) of tRNA, An4Ac1T1V4
  source 1..68: mol_type = other DNA
tggttgcgggggccggatttgaaccgacgacccctgggttatgagcccagtgcgctaccaggctgcgc

SEQ ID NO: 110 - DNA, 68 bp, synthetic construct
  misc_feature 1..68: note = Extension primer (reverse) of tRNA, An4Ac1T2V1
  source 1..68: mol_type = other DNA
tggttgcggggaccggatttgaaccgacgatctctgggttatgagcccagtgcgctaccaggctgcgc

SEQ ID NO: 111 - DNA, 68 bp, synthetic construct
  misc_feature 1..68: note = Extension primer (reverse) of tRNA, An4Ac1T2V2
  source 1..68: mol_type = other DNA
tggttgcggggaccggatttgaaccgacgatccctgggttatgagcccagtgcgctaccaggctgcgc

SEQ ID NO: 112 - DNA, 68 bp, synthetic construct
  misc_feature 1..68: note = Extension primer (reverse) of tRNA, An4Ac1T2V3
  source 1..68: mol_type = other DNA
tggttgcggggaccggatttgaaccgacgacctctgggttatgagcccagtgcgctaccaggctgcgc

SEQ ID NO: 113 - DNA, 68 bp, synthetic construct
  misc_feature 1..68: note = Extension primer (reverse) of tRNA, An4Ac1T2V4
  source 1..68: mol_type = other DNA
tggttgcggggaccggatttgaaccgacgacccctgggttatgagcccagtgcgctaccaggctgcgc

SEQ ID NO: 114 - DNA, 68 bp, synthetic construct
  misc_feature 1..68: note = Extension primer (reverse) of tRNA, An4Ac1T3V1
  source 1..68: mol_type = other DNA
tggttgcggggagcggatttgaaccgccgatctctgggttatgagcccagtgcgctaccaggctgcgc

SEQ ID NO: 115 - DNA, 68 bp, synthetic construct
  misc_feature 1..68: note = Extension primer (reverse) of tRNA, An4Ac1T3V2
  source 1..68: mol_type = other DNA
tggttgcggggagcggatttgaaccgccgatccctgggttatgagcccagtgcgctaccaggctgcgc

SEQ ID NO: 116 - DNA, 68 bp, synthetic construct
  misc_feature 1..68: note = Extension primer (reverse) of tRNA, An4Ac1T3V3 (=iniP)
  source 1..68: mol_type = other DNA
tggttgcggggagcggatttgaaccgccgacctctgggttatgagcccagtgcgctaccaggctgcgc

SEQ ID NO: 117 - DNA, 68 bp, synthetic construct
  misc_feature 1..68: note = Extension primer (reverse) of tRNA, An4Ac1T3V4
  source 1..68: mol_type = other DNA
tggttgcggggagcggatttgaaccgccgacccctgggttatgagcccagtgcgctaccaggctgcgc

SEQ ID NO: 118 - DNA, 68 bp, synthetic construct
  misc_feature 1..68: note = Extension primer (reverse) of tRNA, An4Ac1T4V1
  source 1..68: mol_type = other DNA
tggttgcggggagaggatttgaacctccgatctctgggttatgagcccagtgcgctaccaggctgcgc

SEQ ID NO: 119 - DNA, 68 bp, synthetic construct
  misc_feature 1..68: note = Extension primer (reverse) of tRNA, An4Ac1T4V2
  source 1..68: mol_type = other DNA
tggttgcggggagaggatttgaacctccgatccctgggttatgagcccagtgcgctaccaggctgcgc

SEQ ID NO: 120 - DNA, 68 bp, synthetic construct
  misc_feature 1..68: note = Extension primer (reverse) of tRNA, An4Ac1T4V3
  source 1..68: mol_type = other DNA
tggttgcggggagaggatttgaacctccgacctctgggttatgagcccagtgcgctaccaggctgcgc

SEQ ID NO: 121 - DNA, 68 bp, synthetic construct
  misc_feature 1..68: note = Extension primer (reverse) of tRNA, An4Ac1T4V4
  source 1..68: mol_type = other DNA
tggttgcggggagaggatttgaacctccgacccctgggttatgagcccagtgcgctaccaggctgcgc

SEQ ID NO: 122 - DNA, 68 bp, synthetic construct
  misc_feature 1..68: note = Extension primer (reverse) of tRNA, An4Ac1T3V3, anticodon=CUU
  source 1..68: mol_type = other DNA
tggttgcggggagcggatttgaaccgccgacctctgggttaagagcccagtgcgctaccaggctgcgc

SEQ ID NO: 123 - DNA, 22 bp, synthetic construct
  misc_feature 1..22: note = PCR primer (forward) of tRNA, iniWT
  source 1..22: mol_type = other DNA
ggcgtaatacgactcactatac

SEQ ID NO: 124 - DNA, 22 bp, synthetic construct
  misc_feature 1..22: note = PCR primer (forward) of tRNA, iniC1G
  source 1..22: mol_type = other DNA
ggcgtaatacgactcactatag

SEQ ID NO: 125 - DNA, 22 bp, synthetic construct
  misc_feature 1..22: note = PCR primer (forward) of tRNA, An1Ac1T1V1 (=iniC1G/A11C/U24G)
  source 1..22: mol_type = other DNA
ggcgtaatacgactcactatag

SEQ ID NO: 126 - DNA, 22 bp, synthetic construct
  misc_feature 1..22: note = PCR primer (forward) of tRNA, An2Ac1T1V1
  source 1..22: mol_type = other DNA
ggcgtaatacgactcactatag

SEQ ID NO: 127 - DNA, 22 bp, synthetic construct
  misc_feature 1..22: note = PCR primer (forward) of tRNA, An3Ac1T1V1
  source 1..22: mol_type = other DNA
ggcgtaatacgactcactatag

SEQ ID NO: 128 - DNA, 22 bp, synthetic construct
  misc_feature 1..22: note = PCR primer (forward) of tRNA, An4Ac1T1V1
  source 1..22: mol_type = other DNA
ggcgtaatacgactcactatag

SEQ ID NO: 129 - DNA, 22 bp, synthetic construct
  misc_feature 1..22: note = PCR primer (forward) of tRNA, An5Ac1T1V1
  source 1..22: mol_type = other DNA
ggcgtaatacgactcactatag

SEQ ID NO: 130 - DNA, 22 bp, synthetic construct
  misc_feature 1..22: note = PCR primer (forward) of tRNA, An4Ac2T1V1
  source 1..22: mol_type = other DNA
ggcgtaatacgactcactatag

SEQ ID NO: 131 - DNA, 22 bp, synthetic construct
  misc_feature 1..22: note = PCR primer (forward) of tRNA, An4Ac3T1V1
  source 1..22: mol_type = other DNA
ggcgtaatacgactcactatag

SEQ ID NO: 132 - DNA, 22 bp, synthetic construct
  misc_feature 1..22: note = PCR primer (forward) of tRNA, An4Ac4T1V1
  source 1..22: mol_type = other DNA
ggcgtaatacgactcactatag

SEQ ID NO: 133 - DNA, 22 bp, synthetic construct
  misc_feature 1..22: note = PCR primer (forward) of tRNA, An4Ac5T1V1
  source 1..22: mol_type = other DNA
ggcgtaatacgactcactatag

SEQ ID NO: 134 - DNA, 22 bp, synthetic construct
  misc_feature 1..22: note = PCR primer (forward) of tRNA, An4Ac1T1V2
  source 1..22: mol_type = other DNA
ggcgtaatacgactcactatag

SEQ ID NO: 135 - DNA, 22 bp, synthetic construct
  misc_feature 1..22: note = PCR primer (forward) of tRNA, An4Ac1T1V3
  source 1..22: mol_type = other DNA
ggcgtaatacgactcactatag

SEQ ID NO: 136 - DNA, 22 bp, synthetic construct
  misc_feature 1..22: note = PCR primer (forward) of tRNA, An4Ac1T1V4
  source 1..22: mol_type = other DNA
ggcgtaatacgactcactatag

SEQ ID NO: 137 - DNA, 22 bp, synthetic construct
  misc_feature 1..22: note = PCR primer (forward) of tRNA, An4Ac1T2V1
  source 1..22: mol_type = other DNA
ggcgtaatacgactcactatag

SEQ ID NO: 138 - DNA, 22 bp, synthetic construct
  misc_feature 1..22: note = PCR primer (forward) of tRNA, An4Ac1T2V2
  source 1..22: mol_type = other DNA
ggcgtaatacgactcactatag

SEQ ID NO: 139 - DNA, 22 bp, synthetic construct
  misc_feature 1..22: note = PCR primer (forward) of tRNA, An4Ac1T2V3
  source 1..22: mol_type = other DNA
ggcgtaatacgactcactatag

SEQ ID NO: 140 - DNA, 22 bp, synthetic construct
  misc_feature 1..22: note = PCR primer (forward) of tRNA, An4Ac1T2V4
  source 1..22: mol_type = other DNA
ggcgtaatacgactcactatag

SEQ ID NO: 141 - DNA, 22 bp, synthetic construct
  misc_feature 1..22: note = PCR primer (forward) of tRNA, An4Ac1T3V1
  source 1..22: mol_type = other DNA
ggcgtaatacgactcactatag

SEQ ID NO: 142 - DNA, 22 bp, synthetic construct
  misc_feature 1..22: note = PCR primer (forward) of tRNA, An4Ac1T3V2
  source 1..22: mol_type = other DNA
ggcgtaatacgactcactatag

SEQ ID NO: 143 - DNA, 22 bp, synthetic construct
  misc_feature 1..22: note = PCR primer (forward) of tRNA, An4Ac1T3V3 (=iniP)
  source 1..22: mol_type = other DNA
ggcgtaatacgactcactatag

SEQ ID NO: 144 - DNA, 22 bp, synthetic construct
  misc_feature 1..22: note = PCR primer (forward) of tRNA, An4Ac1T3V4
  source 1..22: mol_type = other DNA
ggcgtaatacgactcactatag

SEQ ID NO: 145 - DNA, 22 bp, synthetic construct
  misc_feature 1..22: note = PCR primer (forward) of tRNA, An4Ac1T4V1
  source 1..22: mol_type = other DNA
ggcgtaatacgactcactatag

SEQ ID NO: 146 - DNA, 22 bp, synthetic construct
  misc_feature 1..22: note = PCR primer (forward) of tRNA, An4Ac1T4V2
  source 1..22: mol_type = other DNA
ggcgtaatacgactcactatag

SEQ ID NO: 147 - DNA, 22 bp, synthetic construct
  misc_feature 1..22: note = PCR primer (forward) of tRNA, An4Ac1T4V3
  source 1..22: mol_type = other DNA
ggcgtaatacgactcactatag

SEQ ID NO: 148 - DNA, 22 bp, synthetic construct
  misc_feature 1..22: note = PCR primer (forward) of tRNA, An4Ac1T4V4
  source 1..22: mol_type = other DNA
ggcgtaatacgactcactatag

SEQ ID NO: 149 - DNA, 22 bp, synthetic construct
  misc_feature 1..22: note = PCR primer (forward) of tRNA, An4Ac1T3V3, anticodon=CUU
  source 1..22: mol_type = other DNA
ggcgtaatacgactcactatag

SEQ ID NO: 150 - DNA, 17 bp, synthetic construct
  misc_feature 1..17: note = PCR primer (reverse) of tRNA, iniWT
  source 1..17: mol_type = other DNA
  modified_base 2: mod_base = gm
tngttgcgggggccgga

SEQ ID NO: 151 - DNA, 17 bp, synthetic construct
  misc_feature 1..17: note = PCR primer (reverse) of tRNA, iniC1G
  source 1..17: mol_type = other DNA
  modified_base 2: mod_base = gm
tngttgcgggggccgga

SEQ ID NO: 152 - DNA, 20 bp, synthetic construct
  misc_feature 1..20: note = PCR primer (reverse) of tRNA, An1Ac1T1V1 (=iniC1G/A11C/U24G)
  source 1..20: mol_type = other DNA
  modified_base 2: mod_base = gm
tngttgcgggggccggattt

SEQ ID NO: 153 - DNA, 20 bp, synthetic construct
  misc_feature 1..20: note = PCR primer (reverse) of tRNA, An2Ac1T1V1
  source 1..20: mol_type = other DNA
  modified_base 2: mod_base = gm
tngttgcgggggccggattt

SEQ ID NO: 154 - DNA, 20 bp, synthetic construct
  misc_feature 1..20: note = PCR primer (reverse) of tRNA, An3Ac1T1V1
  source 1..20: mol_type = other DNA
  modified_base 2: mod_base = gm
tngttgcgggggccggattt

SEQ ID NO: 155 - DNA, 20 bp, synthetic construct
  misc_feature 1..20: note = PCR primer (reverse) of tRNA, An4Ac1T1V1
  source 1..20: mol_type = other DNA
  modified_base 2: mod_base = gm
tngttgcgggggccggattt

SEQ ID NO: 156 - DNA, 20 bp, synthetic construct
  misc_feature 1..20: note = PCR primer (reverse) of tRNA, An5Ac1T1V1
  source 1..20: mol_type = other DNA
  modified_base 2: mod_base = gm
tngttgcgggggccggattt

SEQ ID NO: 157 - DNA, 20 bp, synthetic construct
  misc_feature 1..20: note = PCR primer (reverse) of tRNA, An4Ac2T1V1
  source 1..20: mol_type = other DNA
  modified_base 2: mod_base = gm
tngttgcgggtgccggattt

SEQ ID NO: 158 - DNA, 20 bp, synthetic construct
  misc_feature 1..20: note = PCR primer (reverse) of tRNA, An4Ac3T1V1
  source 1..20: mol_type = other DNA
  modified_base 2: mod_base = gm
tngttgcggatgccggattt

SEQ ID NO: 159 - DNA, 20 bp, synthetic construct
  misc_feature 1..20: note = PCR primer (reverse) of tRNA, An4Ac4T1V1
  source 1..20: mol_type = other DNA
  modified_base 2: mod_base = gm
tngttgctgatgccggattt

SEQ ID NO: 160 - DNA, 20 bp, synthetic construct
  misc_feature 1..20: note = PCR primer (reverse) of tRNA, An4Ac5T1V1
  source 1..20: mol_type = other DNA
  modified_base 2: mod_base = gm
tngttggtgatgccggattt

SEQ ID NO: 161 - DNA, 20 bp, synthetic construct
  misc_feature 1..20: note = PCR primer (reverse) of tRNA, An4Ac1T1V2
  source 1..20: mol_type = other DNA
  modified_base 2: mod_base = gm
tngttgcgggggccggattt

SEQ ID NO: 162 - DNA, 20 bp, synthetic construct
  misc_feature 1..20: note = PCR primer (reverse) of tRNA, An4Ac1T1V3
  source 1..20: mol_type = other DNA
  modified_base 2: mod_base = gm
tngttgcgggggccggattt

SEQ ID NO: 163 - DNA, 20 bp, synthetic construct
  misc_feature 1..20: note = PCR primer (reverse) of tRNA, An4Ac1T1V4
  source 1..20: mol_type = other DNA
  modified_base 2: mod_base = gm
tngttgcgggggccggattt

SEQ ID NO: 164 - DNA, 20 bp, synthetic construct
  misc_feature 1..20: note = PCR primer (reverse) of tRNA, An4Ac1T2V1
  source 1..20: mol_type = other DNA
  modified_base 2: mod_base = gm
tngttgcggggaccggattt

SEQ ID NO: 165 - DNA, 20 bp, synthetic construct
  misc_feature 1..20: note = PCR primer (reverse) of tRNA, An4Ac1T2V2
  source 1..20: mol_type = other DNA
  modified_base 2: mod_base = gm
tngttgcggggaccggattt

SEQ ID NO: 166 - DNA, 20 bp, synthetic construct
  misc_feature 1..20: note = PCR primer (reverse) of tRNA, An4Ac1T2V3
  source 1..20: mol_type = other DNA
  modified_base 2: mod_base = gm
tngttgcggggaccggattt

SEQ ID NO: 167 - DNA, 20 bp, synthetic construct
  misc_feature 1..20: note = PCR primer (reverse) of tRNA, An4Ac1T2V4
  source 1..20: mol_type = other DNA
  modified_base 2: mod_base = gm
tngttgcggggaccggattt

SEQ ID NO: 168 - DNA, 20 bp, synthetic construct
  misc_feature 1..20: note = PCR primer (reverse) of tRNA, An4Ac1T3V1
  source 1..20: mol_type = other DNA
  modified_base 2: mod_base = gm
tngttgcggggagcggattt

SEQ ID NO: 169 - DNA, 20 bp, synthetic construct
  misc_feature 1..20: note = PCR primer (reverse) of tRNA, An4Ac1T3V2
  source 1..20: mol_type = other DNA
  modified_base 2: mod_base = gm
tngttgcggggagcggattt

SEQ ID NO: 170 - DNA, 20 bp, synthetic construct
  misc_feature 1..20: note = PCR primer (reverse) of tRNA, An4Ac1T3V3 (=iniP)
  source 1..20: mol_type = other DNA
  modified_base 2: mod_base = gm
tngttgcggggagcggattt

SEQ ID NO: 171 - DNA, 20 bp, synthetic construct
  misc_feature 1..20: note = PCR primer (reverse) of tRNA, An4Ac1T3V4
  source 1..20: mol_type = other DNA
  modified_base 2: mod_base = gm
tngttgcggggagcggattt

SEQ ID NO: 172 - DNA, 20 bp, synthetic construct
  misc_feature 1..20: note = PCR primer (reverse) of tRNA, An4Ac1T4V1
  source 1..20: mol_type = other DNA
  modified_base 2: mod_base = gm
tngttgcggggagaggattt

SEQ ID NO: 173 - DNA, 20 bp, synthetic construct
  misc_feature 1..20: note = PCR primer (reverse) of tRNA, An4Ac1T4V2
  source 1..20: mol_type = other DNA
  modified_base 2: mod_base = gm
tngttgcggggagaggattt

SEQ ID NO: 174 - DNA, 20 bp, synthetic construct
  misc_feature 1..20: note = PCR primer (reverse) of tRNA, An4Ac1T4V3
  source 1..20: mol_type = other DNA
  modified_base 2: mod_base = gm
tngttgcggggagaggattt

SEQ ID NO: 175 - DNA, 20 bp, synthetic construct
  misc_feature 1..20: note = PCR primer (reverse) of tRNA, An4Ac1T4V4
  source 1..20: mol_type = other DNA
  modified_base 2: mod_base = gm
tngttgcggggagaggattt

SEQ ID NO: 176 - DNA, 20 bp, synthetic construct
  misc_feature 1..20: note = PCR primer (reverse) of tRNA, An4Ac1T3V3, anticodon=CUU
  source 1..20: mol_type = other DNA
  modified_base 2: mod_base = gm
tngttgcggggagcggattt

SEQ ID NO: 177 - RNA, 86 nt, synthetic construct
  misc_feature 1..86: note = RNA sequence of mR1
  source 1..86: mol_type = other RNA
gggttaactttaagaaggagaaaaacatgtactacgactactacgacaagaaggattataaggatgatgatgataagtaagcttcg

SEQ ID NO: 178 - RNA, 89 nt, synthetic construct
  misc_feature 1..89: note = RNA sequence of mR2
  source 1..89: mol_type = other RNA
gggttgaactttaagtaggagatatatccatgtactacgactactacgacaagaaggattataaggatgatgatgataagtaagcttcg

SEQ ID NO: 179 - RNA, 90 nt, synthetic construct
  misc_feature 1..90: note = RNA sequence of mR3
  source 1..90: mol_type = other RNA
gggttgaactttaataaggaggtaggatccatgtactacgactactacgacaagaaggattataaggatgatgatgataagtaagcttcg

SEQ ID NO: 180 - RNA, 89 nt, synthetic construct
  misc_feature 1..89: note = RNA sequence of mR4
  source 1..89: mol_type = other RNA
gggttgaactttaataaggaggtagatccatgtactacgactactacgacaagaaggattataaggatgatgatgataagtaagcttcg

SEQ ID NO: 181 - RNA, 88 nt, synthetic construct
  misc_feature 1..88: note = RNA sequence of mR5
  source 1..88: mol_type = other RNA
gggttgaactttaataaggaggtagatcatgtactacgactactacgacaagaaggattataaggatgatgatgataagtaagcttcg

SEQ ID NO: 182 - RNA, 87 nt, synthetic construct
  misc_feature 1..87: note = RNA sequence of mR6
  source 1..87: mol_type = other RNA
gggttgaactttaataaggaggtagacatgtactacgactactacgacaagaaggattataaggatgatgatgataagtaagcttcg

SEQ ID NO: 183 - RNA, 86 nt, synthetic construct
  misc_feature 1..86: note = RNA sequence of mR1-AAG
  source 1..86: mol_type = other RNA
gggttaactttaagaaggagaaaaacaagtactacgactactacgacaagaaggattataaggatgatgatgataagtaagcttcg

SEQ ID NO: 184 - RNA, 89 nt, synthetic construct
  misc_feature 1..89: note = RNA sequence of mR2-AAG
  source 1..89: mol_type = other RNA
gggttgaactttaagtaggagatatatccaagtactacgactactacgacaagaaggattataaggatgatgatgataagtaagcttcg

SEQ ID NO: 185 - RNA, 90 nt, synthetic construct
  misc_feature 1..90: note = RNA sequence of mR3-AAG
  source 1..90: mol_type = other RNA
gggttgaactttaataaggaggtaggatccaagtactacgactactacgacaagaaggattataaggatgatgatgataagtaagcttcg

SEQ ID NO: 186 - RNA, 89 nt, synthetic construct
  misc_feature 1..89: note = RNA sequence of mR4-AAG
  source 1..89: mol_type = other RNA
gggttgaactttaataaggaggtagatccaagtactacgactactacgacaagaaggattataaggatgatgatgataagtaagcttcg

SEQ ID NO: 187 - RNA, 88 nt, synthetic construct
  misc_feature 1..88: note = RNA sequence of mR5-AAG
  source 1..88: mol_type = other RNA
gggttgaactttaataaggaggtagatcaagtactacgactactacgacaagaaggattataaggatgatgatgataagtaagcttcg

SEQ ID NO: 188 - RNA, 87 nt, synthetic construct
  misc_feature 1..87: note = RNA sequence of mR6-AAG
  source 1..87: mol_type = other RNA
gggttgaactttaataaggaggtagacaagtactacgactactacgacaagaaggattataaggatgatgatgataagtaagcttcg

SEQ ID NO: 189 - DNA, 43 bp, synthetic construct
  misc_feature 1..43: note = Extension primer (forward) of mR1
  source 1..43: mol_type = other DNA
taatacgactcactatagggttaactttaagaaggagaaaaac

SEQ ID NO: 190 - DNA, 46 bp, synthetic construct
  misc_feature 1..46: note = Extension primer (forward) of mR2
  source 1..46: mol_type = other DNA
taatacgactcactatagggttgaactttaagtaggagatatatcc

SEQ ID NO: 191 - DNA, 47 bp, synthetic construct
  misc_feature 1..47: note = Extension primer (forward) of mR3
  source 1..47: mol_type = other DNA
taatacgactcactatagggttgaactttaataaggaggtaggatcc

SEQ ID NO: 192 - DNA, 46 bp, synthetic construct
  misc_feature 1..46: note = Extension primer (forward) of mR4
  source 1..46: mol_type = other DNA
taatacgactcactatagggttgaactttaataaggaggtagatcc

SEQ ID NO: 193 - DNA, 45 bp, synthetic construct
  misc_feature 1..45: note = Extension primer (forward) of mR5
  source 1..45: mol_type = other DNA
taatacgactcactatagggttgaactttaataaggaggtagatc

SEQ ID NO: 194 - DNA, 44 bp, synthetic construct
  misc_feature 1..44: note = Extension primer (forward) of mR6
  source 1..44: mol_type = other DNA
taatacgactcactatagggttgaactttaataaggaggtagac

SEQ ID NO: 195 - DNA, 43 bp, synthetic construct; identical to SEQ ID NO: 189
  misc_feature 1..43: note = Extension primer (forward) of mR1-AAG
  source 1..43: mol_type = other DNA

SEQ ID NO: 196 - DNA, 46 bp, synthetic construct; identical to SEQ ID NO: 190
  misc_feature 1..46: note = Extension primer (forward) of mR2-AAG
  source 1..46: mol_type = other DNA

SEQ ID NO: 197 - DNA, 47 bp, synthetic construct; identical to SEQ ID NO: 191
  misc_feature 1..47: note = Extension primer (forward) of mR3-AAG
  source 1..47: mol_type = other DNA

SEQ ID NO: 198 - DNA, 46 bp, synthetic construct; identical to SEQ ID NO: 192
  misc_feature 1..46: note = Extension primer (forward) of mR4-AAG
  source 1..46: mol_type = other DNA

SEQ ID NO: 199 - DNA, 45 bp, synthetic construct; identical to SEQ ID NO: 193
  misc_feature 1..45: note = Extension primer (forward) of mR5-AAG
  source 1..45: mol_type = other DNA

SEQ ID NO: 200 - DNA, 44 bp, synthetic construct; identical to SEQ ID NO: 194
  misc_feature 1..44: note = Extension primer (forward) of mR6-AAG
  source 1..44: mol_type = other DNA

SEQ ID NO: 201 - DNA, 60 bp, synthetic construct
  misc_feature 1..60: note = Extension primer (reverse) of mR1
  source 1..60: mol_type = other DNA
cttataatccttcttgtcgtagtagtcgtagtacatgtttttctccttcttaaagttaac

SEQ ID NO: 202 - DNA, 63 bp, synthetic construct
  misc_feature 1..63: note = Extension primer (reverse) of mR2
  source 1..63: mol_type = other DNA
cttataatccttcttgtcgtagtagtcgtagtacatggatatatctcctacttaaagttcaac

SEQ ID NO: 203 - DNA, 64 bp, synthetic construct
  misc_feature 1..64: note = Extension primer (reverse) of mR3
  source 1..64: mol_type = other DNA
cttataatccttcttgtcgtagtagtcgtagtacatggatcctacctccttattaaagttcaac

SEQ ID NO: 204 - DNA, 63 bp, synthetic construct
  misc_feature 1..63: note = Extension primer (reverse) of mR4
  source 1..63: mol_type = other DNA
cttataatccttcttgtcgtagtagtcgtagtacatggatctacctccttattaaagttcaac

SEQ ID NO: 205 - DNA, 62 bp, synthetic construct
  misc_feature 1..62: note = Extension primer (reverse) of mR5
  source 1..62: mol_type = other DNA
cttataatccttcttgtcgtagtagtcgtagtacatgatctacctccttattaaagttcaac

SEQ ID NO: 206 - DNA, 61 bp, synthetic construct
  misc_feature 1..61: note = Extension primer (reverse) of mR6
  source 1..61: mol_type = other DNA
cttataatccttcttgtcgtagtagtcgtagtacatgtctacctccttattaaagttcaac

SEQ ID NO: 207 - DNA, 60 bp, synthetic construct
  misc_feature 1..60: note = Extension primer (reverse) of mR1-AAG
  source 1..60: mol_type = other DNA
cttataatccttcttgtcgtagtagtcgtagtacttgtttttctccttcttaaagttaac

SEQ ID NO: 208 - DNA, 63 bp, synthetic construct
  misc_feature 1..63: note = Extension primer (reverse) of mR2-AAG
  source 1..63: mol_type = other DNA
cttataatccttcttgtcgtagtagtcgtagtacttggatatatctcctacttaaagttcaac

SEQ ID NO: 209 - DNA, 64 bp, synthetic construct
  misc_feature 1..64: note = Extension primer (reverse) of mR3-AAG
  source 1..64: mol_type = other DNA
cttataatccttcttgtcgtagtagtcgtagtacttggatcctacctccttattaaagttcaac

SEQ ID NO: 210 - DNA, 63 bp, synthetic construct
  misc_feature 1..63: note = Extension primer (reverse) of mR4-AAG
  source 1..63: mol_type = other DNA
cttataatccttcttgtcgtagtagtcgtagtacttggatctacctccttattaaagttcaac

SEQ ID NO: 211 - DNA, 62 bp, synthetic construct
  misc_feature 1..62: note = Extension primer (reverse) of mR5-AAG
  source 1..62: mol_type = other DNA
cttataatccttcttgtcgtagtagtcgtagtacttgatctacctccttattaaagttcaac

SEQ ID NO: 212 - DNA, 61 bp, synthetic construct
  misc_feature 1..61: note = Extension primer (reverse) of mR6-AAG
  source 1..61: mol_type = other DNA
cttataatccttcttgtcgtagtagtcgtagtacttgtctacctccttattaaagttcaac

SEQ ID NO: 213 - DNA, 22 bp, synthetic construct
  misc_feature 1..22: note = PCR primer (forward) of mR1
  source 1..22: mol_type = other DNA
ggcgtaatacgactcactatag

SEQ ID NO: 214 - DNA, 22 bp, synthetic construct
  misc_feature 1..22: note = PCR primer (forward) of mR2
  source 1..22: mol_type = other DNA
ggcgtaatacgactcactatag

SEQ ID NO: 215 - DNA, 22 bp, synthetic construct
  misc_feature 1..22: note = PCR primer (forward) of mR3
  source 1..22: mol_type = other DNA
ggcgtaatacgactcactatag

SEQ ID NO: 216 - DNA, 22 bp, synthetic construct
  misc_feature 1..22: note = PCR primer (forward) of mR4
  source 1..22: mol_type = other DNA
ggcgtaatacgactcactatag

SEQ ID NO: 217 - DNA, 22 bp, synthetic construct
  misc_feature 1..22: note = PCR primer (forward) of mR5
  source 1..22: mol_type = other DNA
ggcgtaatacgactcactatag

SEQ ID NO: 218 - DNA, 22 bp, synthetic construct
  misc_feature 1..22: note = PCR primer (forward) of mR6
  source 1..22: mol_type = other DNA
ggcgtaatacgactcactatag

SEQ ID NO: 219 - DNA, 22 bp, synthetic construct
  misc_feature 1..22: note = PCR primer (forward) of mR1-AAG
  source 1..22: mol_type = other DNA
ggcgtaatacgactcactatag

SEQ ID NO: 220 - DNA, 22 bp, synthetic construct
  misc_feature 1..22: note = PCR primer (forward) of mR2-AAG
  source 1..22: mol_type = other DNA
ggcgtaatacgactcactatag

SEQ ID NO: 221 - DNA, 22 bp, synthetic construct
  misc_feature 1..22: note = PCR primer (forward) of mR3-AAG
  source 1..22: mol_type = other DNA
ggcgtaatacgactcactatag

SEQ ID NO: 222 - DNA, 22 bp, synthetic construct
  misc_feature 1..22: note = PCR primer (forward) of mR4-AAG
  source 1..22: mol_type = other DNA
ggcgtaatacgactcactatag

SEQ ID NO: 223 - DNA, 22 bp, synthetic construct
  misc_feature 1..22: note = PCR primer (forward) of mR5-AAG
  source 1..22: mol_type = other DNA
ggcgtaatacgactcactatag

SEQ ID NO: 224 - DNA, 22 bp, synthetic construct
  misc_feature 1..22: note = PCR primer (forward) of mR6-AAG
  source 1..22: mol_type = other DNA
ggcgtaatacgactcactatag

SEQ ID NO: 225 - DNA, 51 bp, synthetic construct
  misc_feature 1..51: note = PCR primer (reverse) of mR1
  source 1..51: mol_type = other DNA
cgaagcttacttatcatcatcatccttataatccttcttgtcgtagtagtc

SEQ ID NO: 226 - DNA, 51 bp, synthetic construct; identical to SEQ ID NO: 225
  misc_feature 1..51: note = PCR primer (reverse) of mR2
  source 1..51: mol_type = other DNA

SEQ ID NO: 227 - DNA, 51 bp, synthetic construct; identical to SEQ ID NO: 225
  misc_feature 1..51: note = PCR primer (reverse) of mR3
  source 1..51: mol_type = other DNA

SEQ ID NO: 228 - DNA, 51 bp, synthetic construct; identical to SEQ ID NO: 225
  misc_feature 1..51: note = PCR primer (reverse) of mR4
  source 1..51: mol_type = other DNA

SEQ ID NO: 229 - DNA, 51 bp, synthetic construct; identical to SEQ ID NO: 225
  misc_feature 1..51: note = PCR primer (reverse) of mR5
  source 1..51: mol_type = other DNA

SEQ ID NO: 230 - DNA, 51 bp, synthetic construct; identical to SEQ ID NO: 225
  misc_feature 1..51: note = PCR primer (reverse) of mR6
  source 1..51: mol_type = other DNA

SEQ ID NO: 231 - DNA, 51 bp, synthetic construct; identical to SEQ ID NO: 225
  misc_feature 1..51: note = PCR primer (reverse) of mR1-AAG
  source 1..51: mol_type = other DNA

SEQ ID NO: 232 - DNA, 51 bp, synthetic construct; identical to SEQ ID NO: 225
  misc_feature 1..51: note = PCR primer (reverse) of mR2-AAG
  source 1..51: mol_type = other DNA

SEQ ID NO: 233 - DNA, 51 bp, synthetic construct; identical to SEQ ID NO: 225
  misc_feature 1..51: note = PCR primer (reverse) of mR3-AAG
  source 1..51: mol_type = other DNA

SEQ ID NO: 234 - DNA, 51 bp, synthetic construct; identical to SEQ ID NO: 225
  misc_feature 1..51: note = PCR primer (reverse) of mR4-AAG
  source 1..51: mol_type = other DNA

SEQ ID NO: 235 - DNA, 51 bp, synthetic construct; identical to SEQ ID NO: 225
  misc_feature 1..51: note = PCR primer (reverse) of mR5-AAG
  source 1..51: mol_type = other DNA

SEQ ID NO: 236 - DNA, 51 bp, synthetic construct; identical to SEQ ID NO: 225
  misc_feature 1..51: note = PCR primer (reverse) of mR6-AAG
  source 1..51: mol_type = other DNA

SEQ ID NO: 237 - protein, 17 aa, synthetic construct
  REGION 1..17: note = P1-FLP-AcPro
  SITE 1: note = N-acetyl-L-proline
PYYDYYDKKDYKDDDDK

SEQ ID NO: 238 - protein, 16 aa, synthetic construct
  REGION 1..16: note = P1-RiP
YYDYYDKKDYKDDDDK

SEQ ID NO: 239 - protein, 17 aa, synthetic construct
  REGION 1..17: note = P1-FLP-AcDTrp
  SITE 1: note = N-acetyl-D-tryptophan
WYYDYYDKKDYKDDDDK

SEQ ID NO: 240 - protein, 17 aa, synthetic construct
  REGION 1..17: note = P1-FLP-AcDTyr
  SITE 1: note = N-acetyl-D-tyrosine
YYYDYYDKKDYKDDDDK

SEQ ID NO: 241 - protein, 17 aa, synthetic construct
  REGION 1..17: note = P1-FLP-AcbetaPhg
  SITE 1: note = N-acetyl-L-beta-homophenylglycine
XYYDYYDKKDYKDDDDK

SEQ ID NO: 242 - protein, 17 aa, synthetic construct
  REGION 1..17: note = P1-FLP-Ac3Abz
  SITE 1: note = N-acetyl-3-aminobenzoic acid
XYYDYYDKKDYKDDDDK

SEQ ID NO: 243-248 - skipped (6 entries)